European Patent Application EP 4 317 428 A1, published February 7, 2024. Title: 食品用酵素組成物  ENZYME COMPOSITION FOR FOOD. Applicant: NAGASE CHEMTEX CORPORATION. The sequence listing filed with the application follows.

SEQUENCE LISTING (2 sequences)

SEQ ID NO: 1 - protein, 345 aa, Streptomyces septatus TH-2
MLELNGPLNGPARRSRAVALLATGAALAATLLGTASGAADAVPTTAKTTATTAAAKGHVRTKAGAPAIPVANVKAHLNQLQSIARANNGNRAHGRSGYKASVDYVKGKLDAAGFTTTVQQFSANGATGYNLIADWPGGDTDHVVFAGSHLDSVSAGPGINDNGSGSAGVLEVALAVAREGYKPDKHLRFGWWGAEELGMVGSQNYVDNLSSADRSKIDAYLNFDMIGSPNPGYYVYGYDANLQSLFENWFAAKNIATEVDHEGDGRSDHAPFQNVGIPVGGLFSGADYIKTAEQAQKWGGTAGRAFDACYHRSCDTYANLNDTALGTNTDAIAGAVWSLSGSATS

SEQ ID NO: 2 - DNA, 1038 bp, Streptomyces septatus TH-2
atgcttgaactcaacggaccactcaacggacctgcccggagaagccgcgccgtcgccctcctggccaccggcgcggccctcgccgccaccctcctcggcacggcctccggcgcggccgacgcggtccccaccaccgcgaagaccaccgccaccaccgccgccgccaagggccacgtcaggaccaaggccggcgcgcccgccatccccgtggccaacgtcaaggcccatctcaaccagctccagtcgatagccagggccaacaacggcaaccgcgcgcacggccgcagcggttacaaggcgtccgtcgactatgtgaagggcaagctggacgccgccggattcaccaccaccgtgcagcagttcagcgccaacggcgccaccggctacaacctgatagccgactggcccggcggtgacaccgaccacgtcgtcttcgccggctcgcacctcgactccgtctccgcgggccccggcatcaacgacaacggctccggctccgccggtgtcctcgaagtcgccctcgccgtcgcccgcgagggctacaagcccgacaagcacctgcggttcggctggtggggcgccgaggaactcggcatggtcggctcgcagaactacgtcgacaacctgtcctccgccgaccggtcgaagatcgacgcctatctgaacttcgacatgatcggctcgccgaacccgggctactacgtctacggctacgacgcgaacctccagagcctcttcgagaactggttcgcggcgaagaacatcgccaccgaggtcgaccacgagggcgacggccgctcggaccacgcgcctttccagaacgtcggcatacccgtcggcgggctcttcagcggcgccgactacatcaagaccgccgagcaggcgcagaagtggggcggcacggcgggccgggcgttcgacgcctgctaccaccgctcgtgcgacacgtacgccaacctgaacgacaccgcgctcggcacgaacaccgatgcgatcgcgggtgcggtgtggtcgctgagcggcagcgccacgagctag